European Patent Application EP 4 406 965 A1, published July 31, 2024. Title: 白介素2突变体以及其融合蛋白. Applicant: 信达生物制药(苏州）有限公司. The sequence listing filed with the application follows.

SEQUENCE LISTING (45 sequences)

SEQ ID NO: 1 - protein, 153 aa, synthetic construct
MYRMQLLSCIALSLALVTNSAPTSSSTKKTQLQLEHLLLDLQMILNGINNYKNPKLTRMLTFKFYMPKKATELKHLQCLEEELKPLEEVLNLAQSKNFHLRPRDLISNINVIVLELKGSETTFMCEYADETATIVEFLNRWITFCQSIISTLT

SEQ ID NO: 2 - protein, 133 aa, synthetic construct [sequence omitted]

SEQ ID NO: 3 - protein, 133 aa, synthetic construct
APTSSSTKKTQLQLEHLLLDLQMILNGINNYKNPKLTRMLTFKFYMPKKATELKHLQCLEEELKPLEEVLNLAQSKNFHLRPRDLISNINVIVLELKGSETTFMCEYADETATIVEFLNRWITFSQSIISTLT

SEQ ID NO: 4 - protein, 129 aa, synthetic construct
APASSSTKKTQLQLEHLLLDLQMILNGINNYKNPKLTRMLTFKFYMPKKATELKHLQCLEEELKPLEEVLNLAGDASIHDLISDINVIVLELKGSETTFMCEYADETATIVEFLNRWITFSQSIISTLT

SEQ ID NO: 5 - protein, 10 aa, synthetic construct
GGGGSGGGGS

SEQ ID NO: 6 - protein, 227 aa, synthetic construct
DKTHTCPPCPAPEAAGGPSVFLFPPKPKDTLMISRTPEVTCVVVDVSHEDPEVKFNWYVDGVEVHNAKTKPREEQYNSTYRVVSVLTVLHQDWLNGKEYKCKVSNKALPAPIEKTISKAKGQPREPQVYTLPPCRDELTKNQVSLWCLVKGFYPSDIAVEWESNGQPENNYKTTPPVLDSDGSFFLYSKLTVDKSRWQQGNVFSCSVMHEALHNHYTQKSLSLSPGK

SEQ ID NO: 7 - protein, 366 aa, synthetic construct
APASSSTKKTQLQLEHLLLDLQMILNGINNYKNPKLTRMLTFKFYMPKKATELKHLQCLEEELKPLEEVLNLAGDASIHDLISDINVIVLELKGSETTFMCEYADETATIVEFLNRWITFSQSIISTLTGGGGSGGGGSDKTHTCPPCPAPEAAGGPSVFLFPPKPKDTLMISRTPEVTCVVVDVSHEDPEVKFNWYVDGVEVHNAKTKPREEQYNSTYRVVSVLTVLHQDWLNGKEYKCKVSNKALPAPIEKTISKAKGQPREPQVYTLPPCRDELTKNQVSLWCLVKGFYPSDIAVEWESNGQPENNYKTTPPVLDSDGSFFLYSKLTVDKSRWQQGNVFSCSVMHEALHNHYTQKSLSLSPGK

SEQ ID NO: 8 - protein, 120 aa, synthetic construct
QVQLVQSGAEVKKPGSSVKVSCKASGGTFSSYAISWVRQAPGQGLEWMGLIIPMFDTAGYAQKFQGRVAITVDESTSTAYMELSSLRSEDTAVYYCARAEHSSTGTFDYWGQGTLVTVSS

SEQ ID NO: 9 - protein, 10 aa, synthetic construct
GGTFSSYAIS

SEQ ID NO: 10 - protein, 17 aa, synthetic construct
LIIPMFDTAGYAQKFQG

SEQ ID NO: 11 - protein, 11 aa, synthetic construct
AEHSSTGTFDY

SEQ ID NO: 12 - protein, 227 aa, synthetic construct
DKTHTCPPCPAPEAAGGPSVFLFPPKPKDTLMISRTPEVTCVVVDVSHEDPEVKFNWYVDGVEVHNAKTKPREEQYNSTYRVVSVLTVLHQDWLNGKEYKCKVSNKALPAPIEKTISKAKGQPREPQVCTLPPSRDELTKNQVSLSCAVKGFYPSDIAVEWESNGQPENNYKTTPPVLDSDGSFFLVSKLTVDKSRWQQGNVFSCSVMHEALHNHYTQKSLSLSPGK

SEQ ID NO: 13 - protein, 330 aa, synthetic construct
ASTKGPSVFPLAPSSKSTSGGTAALGCLVKDYFPEPVTVSWNSGALTSGVHTFPAVLQSSGLYSLSSVVTVPSSSLGTQTYICNVNHKPSNTKVDKKVEPKSCDKTHTCPPCPAPEAAGGPSVFLFPPKPKDTLMISRTPEVTCVVVDVSHEDPEVKFNWYVDGVEVHNAKTKPREEQYNSTYRVVSVLTVLHQDWLNGKEYKCKVSNKALPAPIEKTISKAKGQPREPQVCTLPPSRDELTKNQVSLSCAVKGFYPSDIAVEWESNGQPENNYKTTPPVLDSDGSFFLVSKLTVDKSRWQQGNVFSCSVMHEALHNHYTQKSLSLSPGK

SEQ ID NO: 14 - protein, 450 aa, synthetic construct
QVQLVQSGAEVKKPGSSVKVSCKASGGTFSSYAISWVRQAPGQGLEWMGLIIPMFDTAGYAQKFQGRVAITVDESTSTAYMELSSLRSEDTAVYYCARAEHSSTGTFDYWGQGTLVTVSSASTKGPSVFPLAPSSKSTSGGTAALGCLVKDYFPEPVTVSWNSGALTSGVHTFPAVLQSSGLYSLSSVVTVPSSSLGTQTYICNVNHKPSNTKVDKKVEPKSCDKTHTCPPCPAPEAAGGPSVFLFPPKPKDTLMISRTPEVTCVVVDVSHEDPEVKFNWYVDGVEVHNAKTKPREEQYNSTYRVVSVLTVLHQDWLNGKEYKCKVSNKALPAPIEKTISKAKGQPREPQVCTLPPSRDELTKNQVSLSCAVKGFYPSDIAVEWESNGQPENNYKTTPPVLDSDGSFFLVSKLTVDKSRWQQGNVFSCSVMHEALHNHYTQKSLSLSPGK

SEQ ID NO: 15 - protein, 107 aa, synthetic construct
DIQMTQSPSSVSASVGDRVTITCRASQGISSWLAWYQQKPGKAPKLLISAASSLQSGVPSRFSGSGSGTDFTLTISSLQPEDFATYYCQQANHLPFTFGGGTKVEIK

SEQ ID NO: 16 - protein, 11 aa, synthetic construct
RASQGISSWLA

SEQ ID NO: 17 - protein, 7 aa, synthetic construct
AASSLQS

SEQ ID NO: 18 - protein, 9 aa, synthetic construct
QQANHLPFT

SEQ ID NO: 19 - protein, 107 aa, synthetic construct [sequence omitted]

SEQ ID NO: 20 - protein, 214 aa, synthetic construct
DIQMTQSPSSVSASVGDRVTITCRASQGISSWLAWYQQKPGKAPKLLISAASSLQSGVPSRFSGSGSGTDFTLTISSLQPEDFATYYCQQANHLPFTFGGGTKVEIKRTVAAPSVFIFPPSDEQLKSGTASVVCLLNNFYPREAKVQWKVDNALQSGNSQESVTEQDSKDSTYSLSSTLTLSKADYEKHKVYACEVTHQGLSSPVTKSFNRGEC

SEQ ID NO: 21 - protein, 347 aa, synthetic construct
ASTKGPSVFPLAPSSKSTSGGTAALGCLVKDYFPEPVTVSWNSGALTSGVHTFPAVLQSSGLYSLSSVVTVPSSSLGTQTYICNVNHKPSNTKVDKKVEPKSCDKTHTCPPCPAPEAAGGPSVFLFPPKPKDTLMISRTPEVTCVVVDVSHEDPEVKFNWYVDGVEVHNAKTKPREEQYNSTYRVVSVLTVLHQDWLNGKEYKCKVSNKALPAPIEKTISKAKGQPREPQVYTLPPSRDELTKNQVSLTCLVKGFYPSDIAVEWESNGQPENNYKTTPPVLDSDGSFFLYSKLTVDKSRWQQGNVFSCSVMHEALHNHYTQKSLSLSPGKLALALALAIGGFCADCC

SEQ ID NO: 22 - protein, 467 aa, synthetic construct
QVQLVQSGAEVKKPGSSVKVSCKASGGTFSSYAISWVRQAPGQGLEWMGLIIPMFDTAGYAQKFQGRVAITVDESTSTAYMELSSLRSEDTAVYYCARAEHSSTGTFDYWGQGTLVTVSSASTKGPSVFPLAPSSKSTSGGTAALGCLVKDYFPEPVTVSWNSGALTSGVHTFPAVLQSSGLYSLSSVVTVPSSSLGTQTYICNVNHKPSNTKVDKKVEPKSCDKTHTCPPCPAPEAAGGPSVFLFPPKPKDTLMISRTPEVTCVVVDVSHEDPEVKFNWYVDGVEVHNAKTKPREEQYNSTYRVVSVLTVLHQDWLNGKEYKCKVSNKALPAPIEKTISKAKGQPREPQVYTLPPSRDELTKNQVSLTCLVKGFYPSDIAVEWESNGQPENNYKTTPPVLDSDGSFFLYSKLTVDKSRWQQGNVFSCSVMHEALHNHYTQKSLSLSPGKLALALALAIGGFCADCC

SEQ ID NO: 23 - protein, 129 aa, synthetic construct
APASSSTKKTQLQLEHLLLDLQMILNGINNYKNPKLTRMLTFKFYMPKKATELKHLQCLEEELKPLEEVLNLAGDASIHDLISRINVIVLELKGSETTFMCEYADETATIVEFLNRWITFSQSIISTLT

SEQ ID NO: 24 - protein, 366 aa, synthetic construct
APASSSTKKTQLQLEHLLLDLQMILNGINNYKNPKLTRMLTFKFYMPKKATELKHLQCLEEELKPLEEVLNLAGDASIHDLISRINVIVLELKGSETTFMCEYADETATIVEFLNRWITFSQSIISTLTGGGGSGGGGSDKTHTCPPCPAPEAAGGPSVFLFPPKPKDTLMISRTPEVTCVVVDVSHEDPEVKFNWYVDGVEVHNAKTKPREEQYNSTYRVVSVLTVLHQDWLNGKEYKCKVSNKALPAPIEKTISKAKGQPREPQVYTLPPCRDELTKNQVSLWCLVKGFYPSDIAVEWESNGQPENNYKTTPPVLDSDGSFFLYSKLTVDKSRWQQGNVFSCSVMHEALHNHYTQKSLSLSPGK

SEQ ID NO: 25 - protein, 129 aa, synthetic construct
APASSSTKKTQLQLEHLLLDLQMILNGINNYKNPKLTRMLTFKFYMPKKATELKHLQCLEEELKPLEEVLNLAGDASIHDLISRINVIVLELKGSETTFMCEYADETATIVEFLNRWITFSQSIIRTLT

SEQ ID NO: 26 - protein, 366 aa, synthetic construct
APASSSTKKTQLQLEHLLLDLQMILNGINNYKNPKLTRMLTFKFYMPKKATELKHLQCLEEELKPLEEVLNLAGDASIHDLISRINVIVLELKGSETTFMCEYADETATIVEFLNRWITFSQSIIRTLTGGGGSGGGGSDKTHTCPPCPAPEAAGGPSVFLFPPKPKDTLMISRTPEVTCVVVDVSHEDPEVKFNWYVDGVEVHNAKTKPREEQYNSTYRVVSVLTVLHQDWLNGKEYKCKVSNKALPAPIEKTISKAKGQPREPQVYTLPPCRDELTKNQVSLWCLVKGFYPSDIAVEWESNGQPENNYKTTPPVLDSDGSFFLYSKLTVDKSRWQQGNVFSCSVMHEALHNHYTQKSLSLSPGK

SEQ ID NO: 27 - protein, 129 aa, synthetic construct
APASSSTKKTQLQLEHLLLDLQMILNGINNYKNPKLTRMLTAKFYMPKKATELKHLQCLEEELKPLEEVLNLAQSKNFHDLISRINVIVLELKGSETTFMCEYADETATIVEFLNRWITFSQEIISTLT

SEQ ID NO: 28 - protein, 366 aa, synthetic construct
APASSSTKKTQLQLEHLLLDLQMILNGINNYKNPKLTRMLTAKFYMPKKATELKHLQCLEEELKPLEEVLNLAQSKNFHDLISRINVIVLELKGSETTFMCEYADETATIVEFLNRWITFSQEIISTLTGGGGSGGGGSDKTHTCPPCPAPEAAGGPSVFLFPPKPKDTLMISRTPEVTCVVVDVSHEDPEVKFNWYVDGVEVHNAKTKPREEQYNSTYRVVSVLTVLHQDWLNGKEYKCKVSNKALPAPIEKTISKAKGQPREPQVYTLPPCRDELTKNQVSLWCLVKGFYPSDIAVEWESNGQPENNYKTTPPVLDSDGSFFLYSKLTVDKSRWQQGNVFSCSVMHEALHNHYTQKSLSLSPGK

SEQ ID NO: 29 - protein, 129 aa, synthetic construct
APASSSTKKTQLQLEHLLLDLQMILNGINNYKNPKLTRMLTAKFYMPKKATELKHLQCLEEELKPLEEVLNLAGDASIHDLISRINVIVLELKGSETTFMCEYADETATIVEFLNRWITFSQEIISTLT

SEQ ID NO: 30 - protein, 366 aa, synthetic construct
APASSSTKKTQLQLEHLLLDLQMILNGINNYKNPKLTRMLTAKFYMPKKATELKHLQCLEEELKPLEEVLNLAGDASIHDLISRINVIVLELKGSETTFMCEYADETATIVEFLNRWITFSQEIISTLTGGGGSGGGGSDKTHTCPPCPAPEAAGGPSVFLFPPKPKDTLMISRTPEVTCVVVDVSHEDPEVKFNWYVDGVEVHNAKTKPREEQYNSTYRVVSVLTVLHQDWLNGKEYKCKVSNKALPAPIEKTISKAKGQPREPQVYTLPPCRDELTKNQVSLWCLVKGFYPSDIAVEWESNGQPENNYKTTPPVLDSDGSFFLYSKLTVDKSRWQQGNVFSCSVMHEALHNHYTQKSLSLSPGK

SEQ ID NO: 31 - protein, 129 aa, synthetic construct
APASSSTKKTQLQLEHLLLDLQMILNGINNYKNPELTRMLTFKFYMPKKATELKHLQCLEEELKPLEEVLNLAQSKNFHDLISRINVIVLELKGSETTFMCEYADETATIVEFLNRWITFSQEIISTLT

SEQ ID NO: 32 - protein, 366 aa, synthetic construct
APASSSTKKTQLQLEHLLLDLQMILNGINNYKNPELTRMLTFKFYMPKKATELKHLQCLEEELKPLEEVLNLAQSKNFHDLISRINVIVLELKGSETTFMCEYADETATIVEFLNRWITFSQEIISTLTGGGGSGGGGSDKTHTCPPCPAPEAAGGPSVFLFPPKPKDTLMISRTPEVTCVVVDVSHEDPEVKFNWYVDGVEVHNAKTKPREEQYNSTYRVVSVLTVLHQDWLNGKEYKCKVSNKALPAPIEKTISKAKGQPREPQVYTLPPCRDELTKNQVSLWCLVKGFYPSDIAVEWESNGQPENNYKTTPPVLDSDGSFFLYSKLTVDKSRWQQGNVFSCSVMHEALHNHYTQKSLSLSPGK

SEQ ID NO: 33 - protein, 597 aa, synthetic construct
EVQLLESGGGLVQPGGSLRLSCAASGFSFSSYTMSWVRQAPGKGLEWVATISGGGRDIYYPDSVKGRFTISRDNSKNTLYLQMNSLRAEDTAVYYCVLLTGRVYFALDSWGQGTLVTVSSASTKGPSVFPLAPSSKSTSGGTAALGCLVKDYFPEPVTVSWNSGALTSGVHTFPAVLQSSGLYSLSSVVTVPSSSLGTQTYICNVNHKPSNTKVDKKVEPKSCDKTHTCPPCPAPEAAGGPSVFLFPPKPKDTLMISRTPEVTCVVVDVSHEDPEVKFNWYVDGVEVHNAKTKPREEQYNSTYRVVSVLTVLHQDWLNGKEYKCKVSNKALPAPIEKTISKAKGQPREPQVYTLPPCRDELTKNQVSLWCLVKGFYPSDIAVEWESNGQPENNYKTTPPVLDSDGSFFLYSKLTVDKSRWQQGNVFSCSVMHEALHNHYTQKSLSLSPGGGGGSGGGGSGGGGSAPASSSTKKTQLQLEHLLLDLQMILNGINNYKNPKLTRMLTAKFAMPKKATELKHLQCLEEELKPLEEVLNGAQSKNFHLRPRDLISNINVIVLELKGSETTFMCEYADETATIVEFLNRWITFAQSIISTLT

SEQ ID NO: 34 - protein, 218 aa, synthetic construct
DIVMTQSPDSLAVSLGERATINCKASESVDTSDNSFIHWYQQKPGQSPKLLIYRSSTLESGVPDRFSGSGSGTDFTLTISSLQAEDVAVYYCQQNYDVPWTFGQGTKVEIKRTVAAPSVFIFPPSDEQLKSGTASVVCLLNNFYPREAKVQWKVDNALQSGNSQESVTEQDSKDSTYSLSSTLTLSKADYEKHKVYACEVTHQGLSSPVTKSFNRGEC

SEQ ID NO: 35 - protein, 5 aa, synthetic construct
EPKAS

SEQ ID NO: 36 - protein, 232 aa, synthetic construct
EPKASDKTHTCPPCPAPEAAGGPSVFLFPPKPKDTLMISRTPEVTCVVVDVSHEDPEVKFNWYVDGVEVHNAKTKPREEQYNSTYRVVSVLTVLHQDWLNGKEYKCKVSNKALPAPIEKTISKAKGQPREPQVCTLPPSRDELTKNQVSLSCAVKGFYPSDIAVEWESNGQPENNYKTTPPVLDSDGSFFLVSKLTVDKSRWQQGNVFSCSVMHEALHNHYTQKSLSLSPGK

SEQ ID NO: 37 - protein, 370 aa, synthetic construct
APTSSSTKKTQLQLEHLLLDLQMILNGINNYKNPKLTRMLTFKFYMPKKATELKHLQCLEEELKPLEEVLNLAQSKNFHLRPRDLISNINVIVLELKGSETTFMCEYADETATIVEFLNRWITFSQSIISTLTGGGGSGGGGSDKTHTCPPCPAPEAAGGPSVFLFPPKPKDTLMISRTPEVTCVVVDVSHEDPEVKFNWYVDGVEVHNAKTKPREEQYNSTYRVVSVLTVLHQDWLNGKEYKCKVSNKALPAPIEKTISKAKGQPREPQVYTLPPCRDELTKNQVSLWCLVKGFYPSDIAVEWESNGQPENNYKTTPPVLDSDGSFFLYSKLTVDKSRWQQGNVFSCSVMHEALHNHYTQKSLSLSPGK

SEQ ID NO: 38 - protein, 456 aa, synthetic construct
AVNGTSQFTCFYNSRANISCVWSQDGALQDTSCQVHAWPDRRRWNQTCELLPVSQASWACNLILGAPDSQKLTTVDIVTLRVLCREGVRWRVMAIQDFKPFENLRLMAPISLQVVHVETHRCNISWEISQASHYFERHLEFEARTLSPGHTWEEAPLLTLKQKQEWICLETLTPDTQYEFQVRVKPLQGEFTTWSPWSQPLAFRTKPAALGKDTGLNDIFEAQKIEWHEDKTHTCPPCPAPEAAGGPSVFLFPPKPKDTLMISRTPEVTCVVVDVSHEDPEVKFNWYVDGVEVHNAKTKPREEQYNSTYRVVSVLTVLHQDWLNGKEYKCKVSNKALPAPIEKTISKAKGQPREPQVYTLPPCRDELTKNQVSLWCLVKGFYPSDIAVEWESNGQPENNYKTTPPVLDSDGSFFLYSKLTVDKSRWQQGNVFSCSVMHEALHNHYTQKSLSLSPGK

SEQ ID NO: 39 - protein, 481 aa, synthetic construct
LNTTILTPNGNEDTTADFFLTTMPTDSLSVSTLPLPEVQCFVFNVEYMNCTWNSSSEPQPTNLTLHYWYKNSDNDKVQKCSHYLFSEEITSGCQLQKKEIHLYQTFVVQLQDPREPRRQATQMLKLQNLVIPWAPENLTLHKLSESQLELNWNNRFLNHCLEHLVQYRTDWDHSWTEQSVDYRHKFSLPSVDGQKRYTFRVRSRFNPLCGSAQHWSEWSHPIHWGSNTSKENGLNDIFEAQKIEWHEHHHHHHHDKTHTCPPCPAPEAAGGPSVFLFPPKPKDTLMISRTPEVTCVVVDVSHEDPEVKFNWYVDGVEVHNAKTKPREEQYNSTYRVVSVLTVLHQDWLNGKEYKCKVSNKALPAPIEKTISKAKGQPREPQVCTLPPSRDELTKNQVSLSCAVKGFYPSDIAVEWESNGQPENNYKTTPPVLDSDGSFFLVSKLTVDKSRWQQGNVFSCSVMHEALHNRYTQKSLSLSPGK

SEQ ID NO: 40 - protein, 7 aa, synthetic construct
AGDASIH

SEQ ID NO: 41 - protein, 11 aa, synthetic construct
AQSKNFHLRPR

SEQ ID NO: 42 - protein, 7 aa, synthetic construct
AQSKNFH

SEQ ID NO: 43 - protein, 227 aa, synthetic construct
DKTHTCPPCPAPEAAGGPSVFLFPPKPKDTLMISRTPEVTCVVVDVSHEDPEVKFNWYVDGVEVHNAKTKPREEQYNSTYRVVSVLTVLHQDWLNGKEYKCKVSNKALPAPIEKTISKAKGQPREPQVYTLPPSRDELTKNQVSLTCLVKGFYPSDIAVEWESNGQPENNYKTTPPVLDSDGSFFLYSKLTVDKSRWQQGNVFSCSVMHEALHNHYTQKSLSLSPGK

SEQ ID NO: 44 - protein, 227 aa, synthetic construct
DKTHTCPPCPAPELLGGPSVFLFPPKPKDTLMISRTPEVTCVVVDVSHEDPEVKFNWYVDGVEVHNAKTKPREEQYNSTYRVVSVLTVLHQDWLNGKEYKCKVSNKALPAPIEKTISKAKGQPREPQVYTLPPSRDELTKNQVSLTCLVKGFYPSDIAVEWESNGQPENNYKTTPPVLDSDGSFFLYSKLTVDKSRWQQGNVFSCSVMHEALHNHYTQKSLSLSPGK

SEQ ID NO: 45 - protein, 450 aa, synthetic construct
EVQLLESGGGLVQPGGSLRLSCAASGFSFSSYTMSWVRQAPGKGLEWVATISGGGRDIYYPDSVKGRFTISRDNSKNTLYLQMNSLRAEDTAVYYCVLLTGRVYFALDSWGQGTLVTVSSASTKGPSVFPLAPSSKSTSGGTAALGCLVKDYFPEPVTVSWNSGALTSGVHTFPAVLQSSGLYSLSSVVTVPSSSLGTQTYICNVNHKPSNTKVDKKVEPKSCDKTHTCPPCPAPEAAGGPSVFLFPPKPKDTLMISRTPEVTCVVVDVSHEDPEVKFNWYVDGVEVHNAKTKPREEQYNSTYRVVSVLTVLHQDWLNGKEYKCKVSNKALPAPIEKTISKAKGQPREPQVCTLPPSRDELTKNQVSLSCAVKGFYPSDIAVEWESNGQPENNYKTTPPVLDSDGSFFLVSKLTVDKSRWQQGNVFSCSVMHEALHNHYTQKSLSLSPGK